European Patent Specification EP 3 358 002 B1, published August 28, 2024. Title: Microorganisms possessing two genes encoding PHA synthase derived from Aeromonas caviae, and method  for producin PHA by  those microorganisms. Applicant: kaneka. The sequence listing filed with the application follows.

SEQUENCE LISTING (32 sequences)

SEQ ID NO: 1 - protein, 594 aa, Aeromonas caviae
MSQPSYGPLFEALAHYNDKLLAMAKAQTERTAQALLQTNLDDLGQVLEQGSQQPWQLIQAQMNWWQDQLKLMQHTLLKSAGQPSEPVITPERSDRRFKAEAWSEQPIYDYLKQSYLLTARHLLASVDALEGVPQKSRERLRFFTRQYVNAMAPSNFLATNPELLKLTLESDGQNLVRGLALLAEDLERSADQLNIRLTDESAFELGRDLALTPGRVVQRTELYELIQYSPTTETVGKTPVLIVPPFINKYYIMDMRPQNSLVAWLVAQGQTVFMISWRNPGVAQAQIDLDDYVVDGVIAALDGVEAATGEREVHGIGYCIGGTALSLAMGWLAARRQKQRVRTATLFTTLLDFSQPGELGIFIHEPIIAALEAQNEAKGIMDGRQLAVSFSLLRENSLYWNYYIDSYLKGQSPVAFDLLHWNSDSTNVAGKTHNSLLRRLYLENQLVKGELKIRNTRIDLGKVKTPVLLVSAVDDHIALWQGTWQGMKLFGGEQRFLLAESGHIAGIINPPAANKYGFWHNGAEAESPESWLAGATHQGGSWWPEMMGFIQNRDEGSEPVPARVPEEGLAPAPGHYVKVRLNPVFACPTEEDAA

SEQ ID NO: 2 - protein, 589 aa, Cupriavidus necator
MATGKGAAASTQEGKSQPFKVTPGPFDPATWLEWSRQWQGTEGNGHAAASGIPGLDALAGVKIAPAQLGDIQQRYMKDFSALWQAMAEGKAEATGPLHDRRFAGDAWRTNLPYRFAAAFYLLNARALTELADAVEADAKTRQRIRFAISQWVDAMSPANFLATNPEAQRLLIESGGESLRAGVRNMMEDLTRGKISQTDESAFEVGRNVAVTEGAVVFENEYFQLLQYKPLTDKVHARPLLMVPPCINKYYILDLQPESSLVRHVVEQGHTVFLVSWRNPDASMAGSTWDDYIEHAAIRAIEVARDISGQDKINVLGFCVGGTIVSTALAVLAARGEHPAASVTLLTTLLDFADTGILDVFVDEGHVQLREATLGGGAGAPCALLRGLELANTFSFLRPNDLVWNYVVDNYLKGNTPVPFDLLFWNGDATNLPGPWYCWYLRHTYLQNELKVPGKLTVCGVPVDLASIDVPTYIYGSREDHIVPWTAAYASTALLANKLRFVLGASGHIAGVINPPAKNKRSHWTNDALPESPQQWLAGAIEHHGSWWPDWTAWLAGQAGAKRAAPANYGNARYRAIEPAPGRYVKAKA

SEQ ID NO: 3 - DNA, 842 bp, Cupriavidus necator
cccgggcaagtaccttgccgacatctatgcgctggcgcgcacgcgcctggcgcgcgccggctgtaccgaggtctacggcggcgacgcctgcaccgtggccgacgccggtcgcttctactcctatcggcgcgatggcgtgaccggccgcatggccagcctggtctggctggcggactgagcccgccgctgcctcactcgtccttgcccctggccgcctgcgcgcgctcggcttcagccttgcgtcggcggcggccgggcgtgcccatgatgtagagcaccagcgccaccggcgccatgccatacatcaggaaggtggcaacgcctgccaccacgttgtgctcggtgatcgccatcatcagcgccacgtagagccagccaatggccacgatgtacatcaaaaattcatccttctcgcctatgctctggggcctcggcagatgcgagcgctgcataccgtccggtaggtcgggaagcgtgcagtgccgaggcggattcccgcattgacagcgcgtgcgttgcaaggcaacaatggactcaaatgtctcggaatcgctgacgattcccaggtttctccggcaagcatagcgcatggcgtctccatgcgagaatgtcgcgcttgccggataaaaggggagccgctatcggaatggacgcaagccacggccgcagcaggtgcggtcgagggcttccagccagttccagggcagatgtgccggcagaccctcccgctttgggggaggcgcaagccgggtccattcggatagcatctccccatgcaaagtgccggccagggcaatgcccggagccggttcgaatagtgacggcagagagacaatcaaatc

SEQ ID NO: 4 - DNA, 232 bp, Escherichia coli
tgcttctggcgtcaggcagccatcggaagctgtggtatggctgtgcaggtcgtaaatcactgcataattcgtgtcgctcaaggcgcactcccgttctggataatgttttttgcgccgacatcataacggttctggcaaatattctgaaatgagctgttgacaattaatcatcgaactagttaactagtacgcaagttcacagcggataacaatttcacacaggaaacaattg

SEQ ID NO: 5 - DNA, 236 bp, Artificial Sequence
  Artificial promoter sequence
caattgtgcttctggcgtcaggcagccatcggaagctgtggtatggctgtgcaggtcgtaaatcactgcataattcgtgtcgctcaaggcgcactcccgttctggataatgttttttgcgccgacatcataacggttctggcaaatattctgaaatgagctgttgacaattaatcatccggctcgtataatgtgtggaattgtgagcggataacaatttcacacaggaaacaattg

SEQ ID NO: 6 - DNA, 24 bp, Cupriavidus necator
cacgtgcagagagacaatcaaatc

SEQ ID NO: 7 - DNA, 34 bp, Artificial Sequence
  primer
gcgcgcatttaaatgcaagcagttcggcgtggcg

SEQ ID NO: 8 - DNA, 25 bp, Artificial Sequence
  primer
gcttgctcttcctattcagtcaggg

SEQ ID NO: 9 - DNA, 43 bp, Artificial Sequence
  primer
gcagagagacaatcaaatcatgaagacctacgagaacatcgcc

SEQ ID NO: 10 - DNA, 33 bp, Artificial Sequence
  primer
gcgcgcatttaaattcagggaaagcgccgcagg

SEQ ID NO: 11 - DNA, 45 bp, Artificial Sequence
  primer
ccctgactgaataggaagagcaagccccgggcaagtaccttgccg

SEQ ID NO: 12 - DNA, 22 bp, Artificial Sequence
  primer
catgatttgattgtctctctgc

SEQ ID NO: 13 - DNA, 1785 bp, Artificial Sequence
  Artificially mutated gene encoding PHA synthase derived from Aeromonas caviae
atgagccaaccatcttatggcccgctgttcgaggccctggcccactacaatgacaagctgctggccatggccaaggcccagacagagcgcaccgcccaggcgctgctgcagaccaatctggacgatctgggccaggtgctggagcagggcagccagcaaccctggcagctgatccaggcccagatgaactggtggcaggatcagctcaagctgatgcagcacaccctgctcaaaagcgcaggccagccgagcgagccggtgatcaccccggagcgcagcgatcgccgcttcaaggccgaggcctggagcgaacaacccatctatgactacctcaagcagtcctacctgctcaccgccaggcacctgctggcctcggtggatgccctggagggcgtcccccagaagagccgggagcggctgcgtttcttcacccgccagtacgtcagcgccatggcccccagcaacttcctggccaccaaccccgagctgctcaagctgaccctggagtccggcggccagaacctggtgcgcggactggccctcttggccgaggatctggagcgcagcgccgatcagctcaacatccgcctgaccgacgaatccgccttcgagctcgggcgggatctggccctgaccccgggccgggtggtgcagcgcaccgagctctatgagctcattcagtacagcccgactaccgagacggtgggcaagacacctgtgctgatagtgccgcccttcatcaacaagtactacatcatggacatgcggccccagaactccctggtcgcctggctggtcgcccagggccagacggtattcatgatctcctggcgcaacccgggcgtggcccaggcccaaatcgatctcgacgactacgtggtggatggcgtcatcgccgccctggacggcgtggaggcggccaccggcgagcgggaggtgcacggcatcggctactgcatcggcggcaccgccctgtcgctcgccatgggctggctggcggcgcggcgccagaagcagcgggtgcgcaccgccaccctgttcactaccctgctggacttctcccagcccggggagcttggcatcttcatccacgagcccatcatagcggcgctcgaggcgcaaaatgaggccaagggcatcatggacgggcgccagctggcggtctccttcagcctgctgcgggagaacagcctctactggaactactacatcgacagctacctcaagggtcagagcccggtggccttcgatctgctgcactggaacagcgacagcaccaatgtggcgggcaagacccacaacagcctgctgcgccgtctctacctggagaaccagctggtgaagggggagctcaagatccgcaacacccgcatcgatctcggcaaggtgaagacccctgtgctgctggtgtcggcggtggacgatcacatcgccctctggcagggcacctggcagggcatgaagctgtttggcggggagcagcgcttcctcctggcggagtccggccacatcgccggcatcatcaacccgccggccgccaacaagtacggcttctggcacaacggggccgaggccgagagcccggagagctggctggcaggggcgacgcaccagggcggctcctggtggcccgagatgatgggctttatccagaaccgtgacgaagggtcagagcccgtccccgcgcgggtcccggaggaagggctggcccccgcccccggccactatgtcaaggtgcggctcaaccccgtgtttgcctgcccaacagaggaggacgccgcatga

SEQ ID NO: 14 - DNA, 34 bp, Artificial Sequence
  primer
gcgcgcatttaaatcatggcatctacgccgtcgg

SEQ ID NO: 15 - DNA, 38 bp, Artificial Sequence
  primer
actagtatcgatcaattggccttttctgcctgggtcta

SEQ ID NO: 16 - DNA, 38 bp, Artificial Sequence
  primer
caattgatcgatactagtattgcgggcgtttcttcttg

SEQ ID NO: 17 - DNA, 34 bp, Artificial Sequence
  primer
gcgcgcatttaaatacgctggcgcgtttcgtctg

SEQ ID NO: 18 - DNA, 18 bp, Artificial Sequence
  linker sequence
caattgatcgatactagt

SEQ ID NO: 19 - DNA, 44 bp, Artificial Sequence
  primer
ggcccaattgcacgtgctctctctcaatcaaatcatggcgaccg

SEQ ID NO: 20 - DNA, 70 bp, Artificial Sequence
  primer
gcgcgcactagtcggctgccgactggttgaaccaggccggcaggtcaggctcatgccttggctttgacgt

SEQ ID NO: 21 - DNA, 24 bp, Artificial Sequence
  Artificially mutated Shine Dalgarno sequence derived from Cupriavidus necator
cacgtgctctctctcaatcaaatc

SEQ ID NO: 22 - DNA, 20 bp, Artificial Sequence
  primer
gtgcaattggcgcaacgcaa

SEQ ID NO: 23 - DNA, 40 bp, Artificial Sequence
  primer
aacatacgagccggaagcatgtgtaaagcctggggtgcct

SEQ ID NO: 24 - DNA, 21 bp, Artificial Sequence
  primer
atgcttccggctcgtatgttg

SEQ ID NO: 25 - DNA, 23 bp, Artificial Sequence
  primer
gggcaattgtttcctgtgtgaaa

SEQ ID NO: 26 - DNA, 36 bp, Artificial Sequence
  primer
gcgcgccaattgcacgtgcagagagacaatcaaatc

SEQ ID NO: 27 - DNA, 30 bp, Artificial Sequence
  primer
gcggaattcgcgcaacgcaattaatgtgag

SEQ ID NO: 28 - DNA, 32 bp, Artificial Sequence
  primer
gcgcgcgaattccccgggcaagtaccttgccg

SEQ ID NO: 29 - DNA, 21 bp, Artificial Sequence
  primer
catgatttgattgtctctctg

SEQ ID NO: 30 - DNA, 38 bp, Artificial Sequence
  primer
cagagagacaatcaaatcatgagccaaccatcttatgg

SEQ ID NO: 31 - DNA, 70 bp, Artificial Sequence
  primer
gcgcgcactagtcggctgccgactggttgaaccaggccggcaggtcaggctcatgcggcgtcctcctctg

SEQ ID NO: 32 - DNA, 126 bp, Artificial Sequence
  Artificially mutated promoter derived from Escherichia coli
caattggcgcaacgcaattaatgtgagttagctcactcattaggcaccccaggctttacacatgcttccggctcgtatgttgtgtggaattgtgagcggataacaatttcacacaggaaacaattg